European Patent Specification EP 4 067 484 B1, published October 30, 2024. Title: Novel galactoside O-acetyltransferase variant and a method for producing L-glutamic acid using the same. Applicant: CJ CheilJedang Corporation. The sequence listing filed with the application follows.

SEQUENCE LISTING (19 sequences)

SEQ ID NO: 1 - protein, 225 aa, Unknown
  galactoside O-acetyltransferase variant
MDKDFESIEKMSSGDWYVATGAEREEVAQKTALLFHEYNQIGPTDPARTDEILKTVLNPASGTCTIKAPAIIEYGFNTTIGEHVFINFGLTILDIAPVRIGARSMFGPNCQLFTAGHPVDDWEMRSGGWENGAPISIGEDTWLGGNVTVVGGVSIGDRCVIGAGAVVTKDIPDDSIAVGNPARVVRKRDDSRLERSQLPEGTSVDALRILPTKSTGVSENIAERY

SEQ ID NO: 2 - DNA, 678 bp, Unknown
  galactoside O-acetyltransferase variant
atggacaaggactttgaatctatcgagaaaatgagcagcggcgattggtacgtggctaccggcgcagaacgtgaagaagtggcacaaaaaacagcgttacttttccacgaatacaaccaaattggacctacagaccccgcacgaactgacgaaatattaaaaactgtactaaatcctgccagcggaacctgcacgatcaaagcgccggccatcattgaatacggcttcaacaccacgatcggcgagcatgtgttcatcaactttggcctcaccattttagatatcgcgccggttcgcatcggggcacgcagcatgttcggtccaaactgtcagctcttcaccgcaggtcacccggtcgatgactgggaaatgcgctccggtgggtgggaaaatggcgcgcccatttccattggcgaggatacgtggctgggtggaaatgtcaccgtcgttggtggcgtgagcattggcgataggtgtgtgattggcgcgggggccgtggtgaccaaggatattccggatgattctattgctgtgggcaaccctgcgcgagtagtgcggaaacgtgatgatagccggctcgaacgttcgcagctgccagaaggcacttccgtggatgcgttgaggattcttcctacaaaatcgactggggtgtcagaaaatattgccgaaagatattaa

SEQ ID NO: 3 - protein, 225 aa, Unknown
  galactoside O-acetyltransferase
MDKDFESIEKMSSGDWYVATGAEREEVAQKTALLFHEYNQIGPTDPARTDEILKTVLNPASGTCTIKAPAIIEYGFNTTIGEHVFINFGLTILDIAPVRIGARSMLGPNCQLFTAGHPVDDWEMRSGGWENGAPISIGEDTWLGGNVTVVGGVSIGDRCVIGAGAVVTKDIPDDSIAVGNPARVVRKRDDSRLERSQLPEGTSVDALRILPTKSTGVSENIAERY

SEQ ID NO: 4 - DNA, 678 bp, Unknown
  galactoside O-acetyltransferase
atggacaaggactttgaatctatcgagaaaatgagcagcggcgattggtacgtggctaccggcgcagaacgtgaagaagtggcacaaaaaacagcgttacttttccacgaatacaaccaaattggacctacagaccccgcacgaactgacgaaatattaaaaactgtactaaatcctgccagcggaacctgcacgatcaaagcgccggccatcattgaatacggcttcaacaccacgatcggcgagcatgtgttcatcaactttggcctcaccattttagatatcgcgccggttcgcatcggggcacgcagcatgctcggtccaaactgtcagctcttcaccgcaggtcacccggtcgatgactgggaaatgcgctccggtgggtgggaaaatggcgcgcccatttccattggcgaggatacgtggctgggtggaaatgtcaccgtcgttggtggcgtgagcattggcgataggtgtgtgattggcgcgggggccgtggtgaccaaggatattccggatgattctattgctgtgggcaaccctgcgcgagtagtgcggaaacgtgatgatagccggctcgaacgttcgcagctgccagaaggcacttccgtggatgcgttgaggattcttcctacaaaatcgactggggtgtcagaaaatattgccgaaagatattaa

SEQ ID NO: 5 - DNA, 35 bp, Artificial Sequence
  Primer
tcgagctcggtaccctgcaactgaacgcacaatct

SEQ ID NO: 6 - DNA, 20 bp, Artificial Sequence
  Primer
ttggaccgaacatgctgcgt

SEQ ID NO: 7 - DNA, 20 bp, Artificial Sequence
  Primer
acgcagcatgttcggtccaa

SEQ ID NO: 8 - DNA, 35 bp, Artificial Sequence
  Primer
ctctagaggatcccctccaggccgtgtattttgca

SEQ ID NO: 9 - DNA, 20 bp, Artificial Sequence
  Primer
tgcaactgaacgcacaatct

SEQ ID NO: 10 - DNA, 20 bp, Artificial Sequence
  Primer
tccaggccgtgtattttgca

SEQ ID NO: 11 - DNA, 38 bp, Artificial Sequence
  Primer
tgaattcgagctcggtacccttgaacggaattgggtgg

SEQ ID NO: 12 - DNA, 38 bp, Artificial Sequence
  Primer
cccaggtggcatcggtaccttcacccagcgccacgcag

SEQ ID NO: 13 - DNA, 39 bp, Artificial Sequence
  Primer
cgctgggtgaaggtaccgatgccacctgggttggtcaag

SEQ ID NO: 14 - DNA, 38 bp, Artificial Sequence
  Primer
gtcgactctagaggatccccggacaaggaatggagaga

SEQ ID NO: 15 - DNA, 18 bp, Artificial Sequence
  Primer
cttaccgttgttgccctt

SEQ ID NO: 16 - DNA, 19 bp, Artificial Sequence
  Primer
ctccttcacccacatcatt

SEQ ID NO: 17 - protein, 1205 aa, Unknown
  OdhA
MFQQFQKDPKSVDKEWRELFEAQGGPNATPATTEAQPSAPKESAKPAPKAAPAAKAAPRVETKPAAKTAPKAKESSVPQQPKLPEPGQTPIRGIFKSIAKNMDISLEIPTATSVRDMPARLMFENRAMVNDQLKRTRGGKISFTHIIGYAMVKAVMAHPDMNNSYDVIDGKPTLIVPEHINLGLAIDLPQKDGSRALVVAAIKETEKMNFSEFLAAYEDIVTRSRKGKLTMDDYQGVTVSLTNPGGIGTRHSVPRLTKGQGTIIGVGSMDYPAEFQGASEDRLAELGVGKLVTITSTYDHRVIQGAVSGEFLRTMSRLLTDDSFWDEIFDAMNVPYTPMRWAQDVPNTGVDKNTRVMQLIEAYRSRGHLIADTNPLSWVQPGMPVPDHRDLDIETHSLTIWDLDRTFSVGGFGGKETMTLREVLSRLRAAYTLKVGSEYTHILDRDERTWLQDRLEAGMPKPTQAEQKYILQKLNAAEAFENFLQTKYVGQKRFSLEGAEALIPLMDSAIDTAAGQGLDEVVIGMPHRGRLNVLFNIVGKPLASIFNEFEGQMEQGQIGGSGDVKYHLGSEGQHLQMFGDGEIKVSLTANPSHLEAVNPVMEGIVRAKQDYLDKGVDGKTVVPLLLHGDAAFAGLGIVPETINLAKLRGYDVGGTIHIVVNNQIGFTTTPDSSRSMHYATDYAKAFGCPVFHVNGDDPEAVVWVGQLATEYRRRFGKDVFIDLVCYRLRGHNEADDPSMTQPKMYELITGRETVRAQYTEDLLGRGDLSNEDAEAVVRDFHDQMESVFNEVKEGGKKQAEAQTGITGSQKLPHGLETNISREELLELGQAFANTPEGFNYHPRVAPVAKKRVSSVTEGGIDWAWGELLAFGSLANSGRLVRLAGEDSRRGTFTQRHAVAIDPATAEEFNPLHELAQSKGNNGKFLVYNSALTEYAGMGFEYGYSVGNEDSVVAWEAQFGDFANGAQTIIDEYVSSGEAKWGQTSKLILLLPHGYEGQGPDHSSARIERFLQLCAEGSMTVAQPSTPANHFHLLRRHALSDLKRPLVIFTPKSMLRNKAAASAPEDFTEVTKFQSVIDDPNVADAAKVKKVMLVSGKLYYELAKRKEKDGRDDIAIVRIEMLHPIPFNRISEALAGYPNAEEVLFVQDEPANQGPWPFYQEHLPELIPNMPKMRRVSRRAQSSTATGVAKVHQLEEKQLIDEAFEA

SEQ ID NO: 18 - DNA, 3618 bp, Unknown
  odhA
atgttccagcagttccagaaggaccccaagtccgtggacaaggaatggagagaactctttgaggcgcaggggggaccaaatgctacccccgctacaacagaagcacagccttcagcgcccaaggagtctgcgaaaccagcaccaaaggctgcccctgcagccaaggcagcaccgcgcgtagaaaccaagccggccgccaagaccgcccctaaggccaaggagtcctcagtgccacagcaacctaagcttccggagccaggacaaaccccaatcaggggtattttcaagtccatcgcgaagaacatggatatctccctggaaatcccaaccgcaacctcggttcgcgatatgccagctcgcctcatgttcgaaaaccgcgcgatggtcaacgatcagctcaagcgcacccgcggtggcaagatctccttcacccacatcattggctacgccatggtgaaggcagtcatggctcacccggacatgaacaactcctacgacgtcatcgacggcaagccaaccctgatcgtgcctgagcacatcaacctgggccttgccatcgaccttcctcagaaggacggctcccgcgcacttgtcgtagcagccatcaaggaaaccgagaagatgaacttctccgagttcctcgcagcatacgaagacatcgtgacacgctcccgcaagggcaagctcaccatggatgactaccagggcgttaccgtttccttgaccaacccaggtggcatcggtacccgccactctgtcccacgtctgaccaagggccagggcaccatcatcggtgtcggttccatggattacccagcagagttccagggcgcttccgaagaccgccttgcagagctcggcgttggcaagcttgtcaccatcacctccacctacgatcaccgcgtgatccagggtgctgtgtccggtgaattcctgcgtaccatgtctcgcctgctcaccgatgattccttctgggatgagatcttcgacgcaatgaacgttccttacaccccaatgcgttgggcacaggacgttccaaacaccggtgttgataagaacacccgcgtcatgcagctcattgaggcataccgctcccgtggacacctcatcgctgacaccaacccactttcatgggttcagcctggcatgccagttccagaccaccgcgacctcgacatcgagacccacagcctgaccatctgggatctggaccgtaccttcagcgtcggtggcttcggcggcaaggagaccatgaccctgcgcgaggtactgtcccgcctgcgcgctgcctacaccttgaaggtcggctccgaatacacccacatcctggaccgcgacgagcgcacctggctgcaggaccgcctcgaagccggaatgccaaagccaacccaggcagagcagaagtacatcctgcagaagctgaacgccgcagaggctttcgagaacttcctgcagaccaagtacgtcggccagaagcgcttctccctcgaaggtgcagaagctctcatcccactgatggactccgccatcgacaccgccgcaggccagggcctcgacgaagttgtcatcggtatgccacaccgtggtcgcctcaacgtgctgttcaacatcgtgggcaagccactggcatccatcttcaacgagtttgaaggccaaatggagcagggccagatcggtggctccggtgacgtgaagtaccacctcggttccgaaggccagcacctgcagatgttcggcgacggcgagatcaaggtctccctgactgctaacccgtcccacctggaagctgttaacccagtgatggaaggtatcgtccgcgcaaagcaggactacctggacaagggcgtagacggcaagactgttgtgccactgctgctccacggtgacgctgcattcgcaggcctgggcatcgtgccagaaaccatcaacctggctaagctgcgtggctacgacgtcggaggcaccatccacatcgtggtgaacaaccagatcggcttcaccaccaccccagactccagccgctccatgcactacgcaaccgactacgccaaggcattcggctgcccagtcttccacgtcaatggtgatgacccagaggcagttgtctgggttggccagctggcaaccgagtaccgtcgtcgcttcggcaaggacgtcttcatcgacctcgtttgctaccgcctccgcggccacaacgaagctgatgatccttccatgacccagccaaagatgtatgagctcatcaccggccgcgagaccgttcgtgctcagtacaccgaagacctgctcggacgtggagacctctccaacgaagatgcagaagcagtcgtccgcgacttccacgaccagatggaatctgtgttcaacgaagtcaaggaaggcggcaagaagcaggctgaggcacagaccggcatcaccggctcccagaagcttccacacggccttgagaccaacatctcccgtgaagagctcctggaactgggacaggctttcgccaacaccccagaaggcttcaactaccacccacgtgtggctccagttgctaagaagcgcgtctcctctgtcaccgaaggtggcatcgactgggcatggggcgagctcctcgccttcggttccctggctaactccggccgcttggttcgccttgcaggtgaagattcccgccgcggtaccttcacccagcgccacgcagttgccatcgacccagcgaccgctgaagagttcaacccactccacgagcttgcacagtccaagggcaacaacggtaagttcctggtctacaactccgcactgaccgagtacgcaggcatgggcttcgagtacggctactccgtaggaaacgaagactccgtcgttgcatgggaagcacagttcggcgacttcgccaacggcgctcagaccatcatcgatgagtacgtctcctcaggcgaagctaagtggggccagacctccaagctgatccttctgctgcctcacggctacgaaggccagggcccagaccactcttccgcacgtatcgagcgcttcctgcagctgtgcgctgagggttccatgactgttgctcagccatccaccccagcaaaccacttccacctgctgcgtcgtcacgctctgtccgacctgaagcgtccactggttatcttcaccccgaagtccatgctgcgtaacaaggctgctgcctccgcaccagaagacttcactgaggtcaccaagttccaatccgtgatcgacgatccaaacgttgcagatgcagccaaggtgaagaaggtcatgctggtctccggcaagctgtactacgaattggcaaagcgcaaggagaaggacggacgcgacgacatcgcgatcgttcgtatcgaaatgctccacccaattccgttcaaccgcatctccgaggctcttgccggctaccctaacgctgaggaagtcctcttcgttcaggatgagccagcaaaccagggcccatggccgttctaccaggagcacctcccagagctgatcccgaacatgccaaagatgcgccgcgtttcccgccgcgctcagtcctccaccgcaactggtgttgctaaggtgcaccagctggaggagaagcagcttatcgacgaggctttcgaggcttaa

SEQ ID NO: 19 - DNA, 5803 bp, Unknown
  pDCM2
gttcgcttgctgtccataaaaccgcccagtctagctatcgccatgtaagcccactgcaagctacctgctttctctttgcgcttgcgttttcccttgtccagatagcccagtagctgacattcatccggggtcagcaccgtttctgcggactggctttctacgtgttccgcttcctttagcagcccttgcgccctgagtgcttgcggcagcgtgaagctagcttttatcgccattcgccattcaggctgcgcaactgttgggaagggcgatcggtgcgggcctcttcgctattacgccagctggcgaaagggggatgtgctgcaaggcgattaagttgggtaacgccagggttttcccagtcacgacgttgtaaaacgacggccagtgaattcgagctcggtacccggggatcctctagagtcgacctgcaggcatgcaagcttggcgtaatcatggtcatagctgtttcctgtgtgaaattgttatccgctcacaattccacacaacatacgagccggaagcataaagtgtaaagcctggggtgcctaatgagtgagctaactcacattaattgcgttgcgctcactgcccgctttccagtcgggaaacctgtcgtgccagctgcattaatgaatcggccaacgcgcggggagaggcggtttgcgtattgggcgctcttccgcttcctcgctcactgactcgctgcgctcggtcgttcggctgcggcgagcggtatcagctcactcaaaggcggtaatacggttatccacagaatcaggggataacgcaggaaagaacatgtgagcaaaaggccagcaaaaggccaggaaccgtaaaaaggccgcgttgctggcgtttttccataggctccgcccccctgacgagcatcacaaaaatcgacgctcaagtcagaggtggcgaaacccgacaggactataaagataccaggcgtttccccctggaagctccctcgtgcgctctcctgttccgaccctgccgcttaccggatacctgtccgcctttctcccttcgggaagcgtggcgctttctcaatgctcacgctgtaggtatctcagttcggtgtaggtcgttcgctccaagctgggctgtgtgcacgaaccccccgttcagcccgaccgctgcgccttatccggtaactatcgtcttgagtccaacccggtaagacacgacttatcgccactggcagcagccactggtaacaggattagcagagcgaggtatgtaggcggtgctacagagttcttgaagtggtggcctaactacggctacactagaaggacagtatttggtatctgcgctctgctgaagccagttaccttcggaaaaagagttggtagctcttgatccggcaaacaaaccaccgctggtagcggtggtttttttgtttgcaagcagcagattacgcgcagaaaaaaaggatctcaagaagatcctttgatcttttctacggggtctgacgctcagtggaacgaaaactcacgttaagggattttggtcatgagattatcaaaaaggatcttcacctagatccttttggggtgggcgaagaactccagcatgagatccccgcgctggaggatcatccagccctgatagaaacagaagccactggagcacctcaaaaacaccatcatacactaaatcagtaagttggcagcatcacccgacgcactttgcgccgaataaatacctgtgacggaagatcacttcgcagaataaataaatcctggtgtccctgttgataccgggaagccctgggccaacttttggcgaaaatgagacgttgatcggcacgtaagaggttccaactttcaccataatgaaataagatcactaccgggcgtattttttgagttatcgagattttcaggagctgatagaaacagaagccactggagcacctcaaaaacaccatcatacactaaatcagtaagttggcagcatcacccgacgcactttgcgccgaataaatacctgtgacggaagatcacttcgcagaataaataaatcctggtgtccctgttgataccgggaagccctgggccaacttttggcgaaaatgagacgttgatcggcacgtaagaggttccaactttcaccataatgaaataagatcactaccgggcgtattttttgagttatcgagattttcaggagctctttggcatcgtctctcgcctgtcccctcagttcagtaatttcctgcatttgcctgtttccagtcggtagatattccacaaaacagcagggaagcagcgcttttccgctgcataaccctgcttcggggtcattatagcgattttttcggtatatccatcctttttcgcacgatatacaggattttgccaaagggttcgtgtagactttccttggtgtatccaacggcgtcagccgggcaggataggtgaagtaggcccacccgcgagcgggtgttccttcttcactgtcccttattcgcacctggcggtgctcaacgggaatcctgctctgcgaggctggccggctaccgccggcgtaacagatgagggcaagcggatggctgatgaaaccaagccaaccaggaagggcagcccacctatcaaggtgtactgccttccagacgaacgaagagcgattgaggaaaaggcggcggcggccggcatgagcctgtcggcctacctgctggccgtcggccagggctacaaaatcacgggcgtcgtggactatgagcacgtccgcgagggcgtcccggaaaacgattccgaagcccaacctttcatagaaggcggcggtggaatcgaaatctcgtgatggcaggttgggcgtcgcttggtcggtcatttcgaaaaaggttaggaatacggttagccatttgcctgcttttatatagttcantatgggattcacctttatgttgataagaaataaaagaaaatgccaataggatatcggcattttcttttgcgtttttatttgttaactgttaattgtccttgttcaaggatgctgtctttgacaacagatgttttcttgcctttgatgttcagcaggaagctcggcgcaaacgttgattgtttgtctgcgtagaatcctctgtttgtcatatagcttgtaatcacgacattgtttcctttcgcttgaggtacagcgaagtgtgagtaagtaaaggttacatcgttaggcggatcaagatccatttttaacacaaggccagttttgttcagcggcttgtatgggccagttaaagaattagaaacataaccaagcatgtaaatatcgttagacgtaatgccgtcaatcgtcatttttgatccgcgggagtcagtgaacaggtaccatttgccgttcattttaaagacgttcgcgcgttcaatttcatctgttactgtgttagatgcaatcagcggtttcatcacttttttcagtgtgtaatcatcgtttagctcaatcataccgagagcgccgtttgctaactcagccgtgcgttttttatcgctttgcagaagtttttgactttcttgacggaagaatgatgtgcttttgccatagtatgctttgttaaataaagattcttcgccttggtagccatcttcagttccagtgtttgcttcaaatactaagtatttgtggcctttatcttctacgtagtgaggatctctcagcgtatggttgtcgcctgagctgtagttgccttcatcgatgaactgctgtacattttgatacgtttttccgtcaccgtcaaagattgatttataatcctctacaccgttgatgttcaaagagctgtctgatgctgatacgttaacttgtgcagttgtcagtgtttgtttgccgtaatgtttaccggagaaatcagtgtagaataaacggatttttccgtcagatgtaaatgtggctgaacctgaccattcttgtgtttggtcttttaggatagaatcatttgcatcgaatttgtcgctgtctttaaagacgcggccagcgtttttccagctgtcaatagaagtttcgccgactttttgatagaacatgtaaatcgatgtgtcatccgcatttttaggatctccggctaatgcaaagacgatgtggtagccgtgatagtttgcgacagtgccgtcagcgttttgtaatggccagctgtcccaaacgtccaggccttttgcagaagagatatttttaattgtggacgaatcaaattcagaaacttgatatttttcatttttttgctgttcagggatttgcagcatatcatggcgtgtaatatgggaaatgccgtatgtttccttatatggcttttggttcgtttctttcgcaaacgcttgagttgcgcctcctgccagcagtgcggtagtaaaggttaatactgttgcttgttttgcaaactttttgatgttcatcgttcatgtctccttttttatgtactgtgttagcggtctgcttcttccagccctcctgtttgaagatggcaagttagttacgcacaataaaaaaagacctaaaatatgtaaggggtgacgccaaagtatacactttgccctttacacattttaggtcttgcctgctttatcagtaacaaacccgcgcgatttacttttcgacctcattctattagactctcgtttggattgcaactggtctattttcctcttttgtttgatagaaaatcataaaaggatttgcagactacgggcctaaagaactaaaaaatctatctgtttcttttcattctctgtattttttatagtttctgttgcatgggcataaagttgcctttttaatcacaattcagaaaatatcataatatctcatttcactaaataatagtgaacggcaggtatatgtgatgggttaaaaaggatcaccccagagtcccgctcagaagaactcgtcaagaaggcgatagaaggcgatgcgctgcgaatcgggagcggcgataccgtaaagcacgaggaagcggtcagcccattcgccgccaagctcttcagcaatatcacgggtagccaacgctatgtcctgatagcggtccgccacacccagccggccacagtcgatgaatccagaaaagcggccattttccaccatgatattcggcaagcaggcatcgccatgggtcacgacgagatcctcgccgtcgggcatccgcgccttgagcctggcgaacagttcggctggcgcgagcccctgatgctcttcgtccagatcatcctgatcgacaagaccggcttccatccgagtacgtgctcgctcgatgcgatgtttcgcttggtggtcgaatgggcaggtagccggatcaagcgtatgcagccgccgcattgcatcagccatgatggatactttctcggcaggagcaaggtgagatgacaggagatcctgccccggcacttcgcccaatagcagccagtcccttcccgcttcagtgacaacgtcgagacagctgcgcaaggaacgcccgtcgtggccagccacgatagccgcgctgcctcgtcttggagttcattcagggcaccggacaggtcggtcttgacaaaaagaaccgggcgcccctgcgctgacagccggaacacggcggcatcagagcagccgattgtctgttgtgcccagtcatagccgaatagcctctccacccaagcggccggagaacctgcgtgcaatccatcttgttcaatcatgcgaaacgatcctcatcctgtctcttgatcagatcttgatcccctgcgccatcagatccttggcggcaagaaagccatccagtttactttgcagggcttcccaaccttaccagagggcgccccagctggcaattccg